European Patent Application EP 4 201 422 A1, published June 28, 2023. Title: COMPOSITIONS AND METHODS OF CELLULAR IMMUNOTHERAPY. Applicant: CRAGE MEDICAL CO., LIMITED. Application EP, filed April 21, 2017. The sequence listing filed with the application follows.

SEQUENCE LISTING (41 sequences)

SEQ ID NO: 1 - protein, 247 aa, synthetic construct
  REGION 1..247: note = synthetic polypeptide
QVQLQESGGGLVQPGRSLRLSCAASGFTFSSYAMHWVRQAPGKGLEWVSAISGSGGSTYYADSVKGRFTISRDNSKNTLYLQMNSLRAEDTAVYYCAKDRRGSHADAFDVWGQGTLVTVSSGGGGSGGGGSGGGGSQSALTQPPSASGSPGQSVTISCTGTSSDVGGYNYVSWYQQYPGKAPKLLIYGNSNRPSGVPDRFSGSKSGTSASLAITGLQAEDGADYYCQSYDSSLRVVFGGGTKVTVLG

SEQ ID NO: 2 - protein, 247 aa, synthetic construct
  REGION 1..247: note = synthetic polypeptide
QVQLQESGGGLVQPGRSLRLSCAASGFTFSTYAMNWVRQAPGKGLEWVSAISMSGESTYYADSVKGRFTISRDNSKNTLYLQMNSLRAEDTAVYYCAKDRRGSHADAFDVWGQGTLVTVSSGGGGSGGGGSGGGGSQSALTQPPSASGSPGQSVTISCTGTSSDVGGYNYVSWYQQYPGKAPKLLIYGNSNRPSGVPDRFSGSKSGTSASLAITGLQAEDGADYYCQSYDSSLRVVFGGGTKVTVLG

SEQ ID NO: 3 - protein, 247 aa, synthetic construct
  REGION 1..247: note = synthetic polypeptide
QVQLQESGGGLVQPGRSLRLSCAASGFTFSSYAMHWVRQAPGKGLEWVSAISSSGGSTYYADSVKGRFTISRDNSKNTLYLQMNSLRAEDTAVYYCAKDRRGSHADAFDVWGQGTLVTVSSGGGGSGGGGSGGGGSQSALTQPPSASGSPGQSVTISCTGTSSDVGHKFPVSWYQQYPGKAPKLLIYKNLLRPSGVPDRFSGSKSGTSASLAITGLQAEDGADYYCQSYDSSLRVVFGGGTKVTVLG

SEQ ID NO: 4 - protein, 243 aa, synthetic construct
  REGION 1..243: note = synthetic polypeptide
EVQLVQSGAEVKKPGASVKVSCKASGYTFSDYEMHWVRQAPGQGLEWMGAIHPGSGDTAYNQRFKGRVTITADKSTSTAYMELSSLRSEDTAVYYCARFYSYAYWGQGTLVTVSAGGGGSGGGGSGGGGSDIVMTQTPLSLPVTPGEPASISCRSSQSLVHSNGNTYLQWYLQKPGQSPQLLIYKVSNRFSGVPDRFSGSGSGTDFTLKISRVEAEDVGVYYCSQSIYVPYTFGQGTKLEIKR

SEQ ID NO: 5 - protein, 247 aa, synthetic construct
  REGION 1..247: note = synthetic polypeptide
QVQLQESGGGLVQPGRSLRLSCAASGFTFSTYAMTWVRQAPGKGLEWVSSISSSGESTYYADSVKGRFTISRDNSKNTLYLQMNSLRAEDTAVYYCAKDRRGSHADAFDVWGQGTLVTVSSGGGGSGGGGSGGGGSQSALTQPPSASGSPGQSVTISCTGTSSDVGGYNYVSWYQQYPGKAPKLLIYGNSNRPSGVPDRFSGSKSGTSASLAITGLQAEDGADYYCQSYDSSLRVVFGGGTKVTVLG

SEQ ID NO: 6 - protein, 247 aa, synthetic construct
  REGION 1..247: note = synthetic polypeptide
QVQLQESGGGLVQPGRSLRLSCAASGFTFSTYAMAWVRQAPGKGLEWVSEISSSGSRTYYADSVKGRFTISRDNSKNTLYLQMNSLRAEDTAVYYCAKDRRGSHADAFDVWGQGTLVTVSSGGGGSGGGGSGGGGSQSALTQPPSASGSPGQSVTISCTGTSSDVGGYNYVSWYQQYPGKAPKLLIYGNSNRPSGVPDRFSGSKSGTSASLAITGLQAEDGADYYCQSYDSSLRVVFGGGTKVTVLG

SEQ ID NO: 7 - protein, 247 aa, synthetic construct
  REGION 1..247: note = synthetic polypeptide
QVQLQESGGGLVQPGRSLRLSCAASGFTFSSYAMHWVRQAPGKGLEWVSAISSSGGSTYYADSVKGRFTISRDNSKNTLYLQMNSLRAEDTAVYYCAKDRRGSHADAFDVWGQGTLVTVSSGGGGSGGGGSGGGGSQSALTQPPSASGSPGQSVTISCTGTSSDVGLMHNVSWYQQYPGKAPKLLIYKSSSRPSGVPDRFSGSKSGTSASLAITGLQAEDGADYYCQSYDSSLRVVFGGGTKVTVLG

SEQ ID NO: 8 - protein, 243 aa, synthetic construct
  REGION 1..243: note = synthetic polypeptide
DVVMTQSPLSLPVTPGEPASISCRSSQSLVHSNANTYLHWYLQKPGQSPQLLIYKVSNRFSGVPDRFSGSGSGTDFTLKISRVEAEDVGVYYCSQNTHVPPTFGQGTKLEIKRGGGGSGGGGSGGGGSQVQLVQSGAEVKKPGASVKVSCKASGYTFTDYEMHWVRQAPGQGLEWMGALDPKTGDTAYSQKFKGRVTLTADESTSTAYMELSSLRSEDTAVYYCTRFYSYTYWGQGTLVTVSS

SEQ ID NO: 9 - protein, 45 aa, synthetic construct
  REGION 1..45: note = synthetic polypeptide
TTTPAPRPPTPAPTIASQPLSLRPEACRPAAGGAVHTRGLDFACD

SEQ ID NO: 10 - protein, 27 aa, synthetic construct
  REGION 1..27: note = synthetic peptide
FWVLVVVGGVLACYSLLVTVAFIIFWV

SEQ ID NO: 11 - protein, 41 aa, synthetic construct
  REGION 1..41: note = synthetic polypeptide
RSKRSRLLHSDYMNMTPRRPGPTRKHYQPYAPPRDFAAYRS

SEQ ID NO: 12 - protein, 113 aa, synthetic construct
  REGION 1..113: note = synthetic polypeptide
RVKFSRSADAPAYQQGQNQLYNELNLGRREEYDVLDKRRGRDPEMGGKPQRRKNPQEGLYNELQKDKMAEAYSEIGMKGERRRGKGHDGLYQGLSTATKDTYDALHMQALPPR

SEQ ID NO: 13 - protein, 42 aa, synthetic construct
  REGION 1..42: note = synthetic polypeptide
KRGRKKLLYIFKQPFMRPVQTTQEEDGCSCRFPEEEEGGCEL

SEQ ID NO: 14 - protein, 473 aa, synthetic construct
  REGION 1..473: note = synthetic polypeptide
QVQLQESGGGLVQPGRSLRLSCAASGFTFSSYAMHWVRQAPGKGLEWVSAISGSGGSTYYADSVKGRFTISRDNSKNTLYLQMNSLRAEDTAVYYCAKDRRGSHADAFDVWGQGTLVTVSSGGGGSGGGGSGGGGSQSALTQPPSASGSPGQSVTISCTGTSSDVGGYNYVSWYQQYPGKAPKLLIYGNSNRPSGVPDRFSGSKSGTSASLAITGLQAEDGADYYCQSYDSSLRVVFGGGTKVTVLGTTTPAPRPPTPAPTIASQPLSLRPEACRPAAGGAVHTRGLDFACDFWVLVVVGGVLACYSLLVTVAFIIFWVRSKRSRLLHSDYMNMTPRRPGPTRKHYQPYAPPRDFAAYRSRVKFSRSADAPAYQQGQNQLYNELNLGRREEYDVLDKRRGRDPEMGGKPQRRKNPQEGLYNELQKDKMAEAYSEIGMKGERRRGKGHDGLYQGLSTATKDTYDALHMQALPPR

SEQ ID NO: 15 - protein, 515 aa, synthetic construct
  REGION 1..515: note = synthetic polypeptide
QVQLQESGGGLVQPGRSLRLSCAASGFTFSSYAMHWVRQAPGKGLEWVSAISGSGGSTYYADSVKGRFTISRDNSKNTLYLQMNSLRAEDTAVYYCAKDRRGSHADAFDVWGQGTLVTVSSGGGGSGGGGSGGGGSQSALTQPPSASGSPGQSVTISCTGTSSDVGGYNYVSWYQQYPGKAPKLLIYGNSNRPSGVPDRFSGSKSGTSASLAITGLQAEDGADYYCQSYDSSLRVVFGGGTKVTVLGTTTPAPRPPTPAPTIASQPLSLRPEACRPAAGGAVHTRGLDFACDFWVLVVVGGVLACYSLLVTVAFIIFWVRSKRSRLLHSDYMNMTPRRPGPTRKHYQPYAPPRDFAAYRSKRGRKKLLYIFKQPFMRPVQTTQEEDGCSCRFPEEEEGGCELRVKFSRSADAPAYQQGQNQLYNELNLGRREEYDVLDKRRGRDPEMGGKPQRRKNPQEGLYNELQKDKMAEAYSEIGMKGERRRGKGHDGLYQGLSTATKDTYDALHMQALPPR

SEQ ID NO: 16 - protein, 515 aa, synthetic construct
  REGION 1..515: note = synthetic polypeptide
QVQLQESGGGLVQPGRSLRLSCAASGFTFSTYAMTWVRQAPGKGLEWVSSISSSGESTYYADSVKGRFTISRDNSKNTLYLQMNSLRAEDTAVYYCAKDRRGSHADAFDVWGQGTLVTVSSGGGGSGGGGSGGGGSQSALTQPPSASGSPGQSVTISCTGTSSDVGGYNYVSWYQQYPGKAPKLLIYGNSNRPSGVPDRFSGSKSGTSASLAITGLQAEDGADYYCQSYDSSLRVVFGGGTKVTVLGTTTPAPRPPTPAPTIASQPLSLRPEACRPAAGGAVHTRGLDFACDFWVLVVVGGVLACYSLLVTVAFIIFWVRSKRSRLLHSDYMNMTPRRPGPTRKHYQPYAPPRDFAAYRSKRGRKKLLYIFKQPFMRPVQTTQEEDGCSCRFPEEEEGGCELRVKFSRSADAPAYQQGQNQLYNELNLGRREEYDVLDKRRGRDPEMGGKPQRRKNPQEGLYNELQKDKMAEAYSEIGMKGERRRGKGHDGLYQGLSTATKDTYDALHMQALPPR

SEQ ID NO: 17 - protein, 473 aa, synthetic construct
  REGION 1..473: note = synthetic polypeptide
QVQLQESGGGLVQPGRSLRLSCAASGFTFSTYAMTWVRQAPGKGLEWVSSISSSGESTYYADSVKGRFTISRDNSKNTLYLQMNSLRAEDTAVYYCAKDRRGSHADAFDVWGQGTLVTVSSGGGGSGGGGSGGGGSQSALTQPPSASGSPGQSVTISCTGTSSDVGGYNYVSWYQQYPGKAPKLLIYGNSNRPSGVPDRFSGSKSGTSASLAITGLQAEDGADYYCQSYDSSLRVVFGGGTKVTVLGTTTPAPRPPTPAPTIASQPLSLRPEACRPAAGGAVHTRGLDFACDFWVLVVVGGVLACYSLLVTVAFIIFWVRSKRSRLLHSDYMNMTPRRPGPTRKHYQPYAPPRDFAAYRSRVKFSRSADAPAYQQGQNQLYNELNLGRREEYDVLDKRRGRDPEMGGKPQRRKNPQEGLYNELQKDKMAEAYSEIGMKGERRRGKGHDGLYQGLSTATKDTYDALHMQALPPR

SEQ ID NO: 18 - protein, 515 aa, synthetic construct
  REGION 1..515: note = synthetic polypeptide
QVQLQESGGGLVQPGRSLRLSCAASGFTFSTYAMAWVRQAPGKGLEWVSEISSSGSRTYYADSVKGRFTISRDNSKNTLYLQMNSLRAEDTAVYYCAKDRRGSHADAFDVWGQGTLVTVSSGGGGSGGGGSGGGGSQSALTQPPSASGSPGQSVTISCTGTSSDVGGYNYVSWYQQYPGKAPKLLIYGNSNRPSGVPDRFSGSKSGTSASLAITGLQAEDGADYYCQSYDSSLRVVFGGGTKVTVLGTTTPAPRPPTPAPTIASQPLSLRPEACRPAAGGAVHTRGLDFACDFWVLVVVGGVLACYSLLVTVAFIIFWVRSKRSRLLHSDYMNMTPRRPGPTRKHYQPYAPPRDFAAYRSKRGRKKLLYIFKQPFMRPVQTTQEEDGCSCRFPEEEEGGCELRVKFSRSADAPAYQQGQNQLYNELNLGRREEYDVLDKRRGRDPEMGGKPQRRKNPQEGLYNELQKDKMAEAYSEIGMKGERRRGKGHDGLYQGLSTATKDTYDALHMQALPPR

SEQ ID NO: 19 - protein, 473 aa, synthetic construct
  REGION 1..473: note = synthetic polypeptide
QVQLQESGGGLVQPGRSLRLSCAASGFTFSTYAMAWVRQAPGKGLEWVSEISSSGSRTYYADSVKGRFTISRDNSKNTLYLQMNSLRAEDTAVYYCAKDRRGSHADAFDVWGQGTLVTVSSGGGGSGGGGSGGGGSQSALTQPPSASGSPGQSVTISCTGTSSDVGGYNYVSWYQQYPGKAPKLLIYGNSNRPSGVPDRFSGSKSGTSASLAITGLQAEDGADYYCQSYDSSLRVVFGGGTKVTVLGTTTPAPRPPTPAPTIASQPLSLRPEACRPAAGGAVHTRGLDFACDFWVLVVVGGVLACYSLLVTVAFIIFWVRSKRSRLLHSDYMNMTPRRPGPTRKHYQPYAPPRDFAAYRSRVKFSRSADAPAYQQGQNQLYNELNLGRREEYDVLDKRRGRDPEMGGKPQRRKNPQEGLYNELQKDKMAEAYSEIGMKGERRRGKGHDGLYQGLSTATKDTYDALHMQALPPR

SEQ ID NO: 20 - protein, 515 aa, synthetic construct
  REGION 1..515: note = synthetic polypeptide
QVQLQESGGGLVQPGRSLRLSCAASGFTFSTYAMNWVRQAPGKGLEWVSAISMSGESTYYADSVKGRFTISRDNSKNTLYLQMNSLRAEDTAVYYCAKDRRGSHADAFDVWGQGTLVTVSSGGGGSGGGGSGGGGSQSALTQPPSASGSPGQSVTISCTGTSSDVGGYNYVSWYQQYPGKAPKLLIYGNSNRPSGVPDRFSGSKSGTSASLAITGLQAEDGADYYCQSYDSSLRVVFGGGTKVTVLGTTTPAPRPPTPAPTIASQPLSLRPEACRPAAGGAVHTRGLDFACDFWVLVVVGGVLACYSLLVTVAFIIFWVRSKRSRLLHSDYMNMTPRRPGPTRKHYQPYAPPRDFAAYRSKRGRKKLLYIFKQPFMRPVQTTQEEDGCSCRFPEEEEGGCELRVKFSRSADAPAYQQGQNQLYNELNLGRREEYDVLDKRRGRDPEMGGKPQRRKNPQEGLYNELQKDKMAEAYSEIGMKGERRRGKGHDGLYQGLSTATKDTYDALHMQALPPR

SEQ ID NO: 21 - protein, 473 aa, synthetic construct
  REGION 1..473: note = synthetic polypeptide
QVQLQESGGGLVQPGRSLRLSCAASGFTFSTYAMNWVRQAPGKGLEWVSAISMSGESTYYADSVKGRFTISRDNSKNTLYLQMNSLRAEDTAVYYCAKDRRGSHADAFDVWGQGTLVTVSSGGGGSGGGGSGGGGSQSALTQPPSASGSPGQSVTISCTGTSSDVGGYNYVSWYQQYPGKAPKLLIYGNSNRPSGVPDRFSGSKSGTSASLAITGLQAEDGADYYCQSYDSSLRVVFGGGTKVTVLGTTTPAPRPPTPAPTIASQPLSLRPEACRPAAGGAVHTRGLDFACDFWVLVVVGGVLACYSLLVTVAFIIFWVRSKRSRLLHSDYMNMTPRRPGPTRKHYQPYAPPRDFAAYRSRVKFSRSADAPAYQQGQNQLYNELNLGRREEYDVLDKRRGRDPEMGGKPQRRKNPQEGLYNELQKDKMAEAYSEIGMKGERRRGKGHDGLYQGLSTATKDTYDALHMQALPPR

SEQ ID NO: 22 - protein, 515 aa, synthetic construct
  REGION 1..515: note = synthetic polypeptide
QVQLQESGGGLVQPGRSLRLSCAASGFTFSSYAMHWVRQAPGKGLEWVSAISSSGGSTYYADSVKGRFTISRDNSKNTLYLQMNSLRAEDTAVYYCAKDRRGSHADAFDVWGQGTLVTVSSGGGGSGGGGSGGGGSQSALTQPPSASGSPGQSVTISCTGTSSDVGHKFPVSWYQQYPGKAPKLLIYKNLLRPSGVPDRFSGSKSGTSASLAITGLQAEDGADYYCQSYDSSLRVVFGGGTKVTVLGTTTPAPRPPTPAPTIASQPLSLRPEACRPAAGGAVHTRGLDFACDFWVLVVVGGVLACYSLLVTVAFIIFWVRSKRSRLLHSDYMNMTPRRPGPTRKHYQPYAPPRDFAAYRSKRGRKKLLYIFKQPFMRPVQTTQEEDGCSCRFPEEEEGGCELRVKFSRSADAPAYQQGQNQLYNELNLGRREEYDVLDKRRGRDPEMGGKPQRRKNPQEGLYNELQKDKMAEAYSEIGMKGERRRGKGHDGLYQGLSTATKDTYDALHMQALPPR

SEQ ID NO: 23 - protein, 473 aa, synthetic construct
  REGION 1..473: note = synthetic polypeptide
QVQLQESGGGLVQPGRSLRLSCAASGFTFSSYAMHWVRQAPGKGLEWVSAISSSGGSTYYADSVKGRFTISRDNSKNTLYLQMNSLRAEDTAVYYCAKDRRGSHADAFDVWGQGTLVTVSSGGGGSGGGGSGGGGSQSALTQPPSASGSPGQSVTISCTGTSSDVGHKFPVSWYQQYPGKAPKLLIYKNLLRPSGVPDRFSGSKSGTSASLAITGLQAEDGADYYCQSYDSSLRVVFGGGTKVTVLGTTTPAPRPPTPAPTIASQPLSLRPEACRPAAGGAVHTRGLDFACDFWVLVVVGGVLACYSLLVTVAFIIFWVRSKRSRLLHSDYMNMTPRRPGPTRKHYQPYAPPRDFAAYRSRVKFSRSADAPAYQQGQNQLYNELNLGRREEYDVLDKRRGRDPEMGGKPQRRKNPQEGLYNELQKDKMAEAYSEIGMKGERRRGKGHDGLYQGLSTATKDTYDALHMQALPPR

SEQ ID NO: 24 - protein, 515 aa, synthetic construct
  REGION 1..515: note = synthetic polypeptide
QVQLQESGGGLVQPGRSLRLSCAASGFTFSSYAMHWVRQAPGKGLEWVSAISSSGGSTYYADSVKGRFTISRDNSKNTLYLQMNSLRAEDTAVYYCAKDRRGSHADAFDVWGQGTLVTVSSGGGGSGGGGSGGGGSQSALTQPPSASGSPGQSVTISCTGTSSDVGLMHNVSWYQQYPGKAPKLLIYKSSSRPSGVPDRFSGSKSGTSASLAITGLQAEDGADYYCQSYDSSLRVVFGGGTKVTVLGTTTPAPRPPTPAPTIASQPLSLRPEACRPAAGGAVHTRGLDFACDFWVLVVVGGVLACYSLLVTVAFIIFWVRSKRSRLLHSDYMNMTPRRPGPTRKHYQPYAPPRDFAAYRSKRGRKKLLYIFKQPFMRPVQTTQEEDGCSCRFPEEEEGGCELRVKFSRSADAPAYQQGQNQLYNELNLGRREEYDVLDKRRGRDPEMGGKPQRRKNPQEGLYNELQKDKMAEAYSEIGMKGERRRGKGHDGLYQGLSTATKDTYDALHMQALPPR

SEQ ID NO: 25 - protein, 473 aa, synthetic construct
  REGION 1..473: note = synthetic polypeptide
QVQLQESGGGLVQPGRSLRLSCAASGFTFSSYAMHWVRQAPGKGLEWVSAISSSGGSTYYADSVKGRFTISRDNSKNTLYLQMNSLRAEDTAVYYCAKDRRGSHADAFDVWGQGTLVTVSSGGGGSGGGGSGGGGSQSALTQPPSASGSPGQSVTISCTGTSSDVGLMHNVSWYQQYPGKAPKLLIYKSSSRPSGVPDRFSGSKSGTSASLAITGLQAEDGADYYCQSYDSSLRVVFGGGTKVTVLGTTTPAPRPPTPAPTIASQPLSLRPEACRPAAGGAVHTRGLDFACDFWVLVVVGGVLACYSLLVTVAFIIFWVRSKRSRLLHSDYMNMTPRRPGPTRKHYQPYAPPRDFAAYRSRVKFSRSADAPAYQQGQNQLYNELNLGRREEYDVLDKRRGRDPEMGGKPQRRKNPQEGLYNELQKDKMAEAYSEIGMKGERRRGKGHDGLYQGLSTATKDTYDALHMQALPPR

SEQ ID NO: 26 - protein, 469 aa, synthetic construct
  REGION 1..469: note = synthetic polypeptide
DVVMTQSPLSLPVTPGEPASISCRSSQSLVHSNANTYLHWYLQKPGQSPQLLIYKVSNRFSGVPDRFSGSGSGTDFTLKISRVEAEDVGVYYCSQNTHVPPTFGQGTKLEIKRGGGGSGGGGSGGGGSQVQLVQSGAEVKKPGASVKVSCKASGYTFTDYEMHWVRQAPGQGLEWMGALDPKTGDTAYSQKFKGRVTLTADESTSTAYMELSSLRSEDTAVYYCTRFYSYTYWGQGTLVTVSSTTTPAPRPPTPAPTIASQPLSLRPEACRPAAGGAVHTRGLDFACDFWVLVVVGGVLACYSLLVTVAFIIFWVRSKRSRLLHSDYMNMTPRRPGPTRKHYQPYAPPRDFAAYRSRVKFSRSADAPAYQQGQNQLYNELNLGRREEYDVLDKRRGRDPEMGGKPQRRKNPQEGLYNELQKDKMAEAYSEIGMKGERRRGKGHDGLYQGLSTATKDTYDALHMQALPPR

SEQ ID NO: 27 - protein, 511 aa, synthetic construct
  REGION 1..511: note = synthetic polypeptide
DVVMTQSPLSLPVTPGEPASISCRSSQSLVHSNANTYLHWYLQKPGQSPQLLIYKVSNRFSGVPDRFSGSGSGTDFTLKISRVEAEDVGVYYCSQNTHVPPTFGQGTKLEIKRGGGGSGGGGSGGGGSQVQLVQSGAEVKKPGASVKVSCKASGYTFTDYEMHWVRQAPGQGLEWMGALDPKTGDTAYSQKFKGRVTLTADESTSTAYMELSSLRSEDTAVYYCTRFYSYTYWGQGTLVTVSSTTTPAPRPPTPAPTIASQPLSLRPEACRPAAGGAVHTRGLDFACDFWVLVVVGGVLACYSLLVTVAFIIFWVRSKRSRLLHSDYMNMTPRRPGPTRKHYQPYAPPRDFAAYRSKRGRKKLLYIFKQPFMRPVQTTQEEDGCSCRFPEEEEGGCELRVKFSRSADAPAYQQGQNQLYNELNLGRREEYDVLDKRRGRDPEMGGKPQRRKNPQEGLYNELQKDKMAEAYSEIGMKGERRRGKGHDGLYQGLSTATKDTYDALHMQALPPR

SEQ ID NO: 28 - protein, 469 aa, synthetic construct
  REGION 1..469: note = synthetic polypeptide
EVQLVQSGAEVKKPGASVKVSCKASGYTFSDYEMHWVRQAPGQGLEWMGAIHPGSGDTAYNQRFKGRVTITADKSTSTAYMELSSLRSEDTAVYYCARFYSYAYWGQGTLVTVSAGGGGSGGGGSGGGGSDIVMTQTPLSLPVTPGEPASISCRSSQSLVHSNGNTYLQWYLQKPGQSPQLLIYKVSNRFSGVPDRFSGSGSGTDFTLKISRVEAEDVGVYYCSQSIYVPYTFGQGTKLEIKRTTTPAPRPPTPAPTIASQPLSLRPEACRPAAGGAVHTRGLDFACDFWVLVVVGGVLACYSLLVTVAFIIFWVRSKRSRLLHSDYMNMTPRRPGPTRKHYQPYAPPRDFAAYRSRVKFSRSADAPAYQQGQNQLYNELNLGRREEYDVLDKRRGRDPEMGGKPQRRKNPQEGLYNELQKDKMAEAYSEIGMKGERRRGKGHDGLYQGLSTATKDTYDALHMQALPPR

SEQ ID NO: 29 - protein, 466 aa, synthetic construct
  REGION 1..466: note = synthetic polypeptide
EVQLVQSGAEVKKPGASVKVSCKASGYTFSDYEMHWVRQAPGQGLEWMGAIHPGSGDTAYNQRFKGRVTITADKSTSTAYMELSSLRSEDTAVYYCARFYSYAYWGQGTLVTVSAGGGGSGGGGSGGGGSDIVMTQTPLSLPVTPGEPASISCRSSQSLVHSNGNTYLQWYLQKPGQSPQLLIYKVSNRFSGVPDRFSGSGSGTDFTLKISRVEAEDVGVYYCSQSIYVPYTFGQGTKLEIKRTTTPAPRPPTPAPTIASQPLSLRPEACRPAAGGAVHTRGLDFACDIYIWAPLAGTCGVLLLSLVITLYCKRGRKKLLYIFKQPFMRPVQTTQEEDGCSCRFPEEEEGGCELRVKFSRSADAPAYKQGQNQLYNELNLGRREEYDVLDKRRGRDPEMGGKPRRKNPQEGLYNELQKDKMAEAYSEIGMKGERRRGKGHDGLYQGLSTATKDTYDALHMQALPPR

SEQ ID NO: 30 - protein, 511 aa, synthetic construct
  REGION 1..511: note = synthetic polypeptide
EVQLVQSGAEVKKPGASVKVSCKASGYTFSDYEMHWVRQAPGQGLEWMGAIHPGSGDTAYNQRFKGRVTITADKSTSTAYMELSSLRSEDTAVYYCARFYSYAYWGQGTLVTVSAGGGGSGGGGSGGGGSDIVMTQTPLSLPVTPGEPASISCRSSQSLVHSNGNTYLQWYLQKPGQSPQLLIYKVSNRFSGVPDRFSGSGSGTDFTLKISRVEAEDVGVYYCSQSIYVPYTFGQGTKLEIKRTTTPAPRPPTPAPTIASQPLSLRPEACRPAAGGAVHTRGLDFACDFWVLVVVGGVLACYSLLVTVAFIIFWVRSKRSRLLHSDYMNMTPRRPGPTRKHYQPYAPPRDFAAYRSKRGRKKLLYIFKQPFMRPVQTTQEEDGCSCRFPEEEEGGCELRVKFSRSADAPAYQQGQNQLYNELNLGRREEYDVLDKRRGRDPEMGGKPQRRKNPQEGLYNELQKDKMAEAYSEIGMKGERRRGKGHDGLYQGLSTATKDTYDALHMQALPPR

SEQ ID NO: 31 - DNA, 22 bp, synthetic construct
  misc_feature 1..22: note = synthetic primer
  source 1..22: mol_type = other DNA
gcaggggaaagaatagtagaca

SEQ ID NO: 32 - DNA, 18 bp, synthetic construct
  misc_feature 1..18: note = synthetic primer
  source 1..18: mol_type = other DNA
cggcctggcggcgtggag

SEQ ID NO: 33 - DNA, 442 bp, synthetic construct
  misc_feature 1..442: note = synthetic polynucleotide
  source 1..442: mol_type = other DNA
gcaggggaaagaatagtagacataatagcaacagacatacaaactaaagaattacaaaaacaaattacaaaaattcaaaattttatcgatggctccggtgcccgtcagtgggcagagcgcacatcgcccacagtccccgagaagttggggggaggggtcggcaattgaaccggtgcctagagaaggtggcgcggggtaaactgggaaagtgatgtcgtgtactggctccgcctttttcccgagggtgggggagaaccgtatataagtgcagtagtcgccgtgaacgttctttttcgcaacgggtttgccgccagaacacaggtgtcgtgacgcggatccaggcctaagcttacgcgtcctagcgctaccggtcgccaccatggccttaccagtgaccgccttgctcctgccgctggccttgctgctccacgccgccaggccg

SEQ ID NO: 34 - DNA, 36 bp, synthetic construct
  misc_feature 1..36: note = synthetic primer
  source 1..36: mol_type = other DNA
ctccacgccgccaggccggaggtgcagctggtgcag

SEQ ID NO: 35 - DNA, 45 bp, synthetic construct
  misc_feature 1..45: note = synthetic primer
  source 1..45: mol_type = other DNA
gcggtgtcctcgctccgcaggctgctcagctccatgtaggcggtg

SEQ ID NO: 36 - DNA, 49 bp, synthetic construct
  misc_feature 1..49: note = synthetic primer
  source 1..49: mol_type = other DNA
gcggagcgaggacaccgccgtgtactactgcgcccggttctacagctac

SEQ ID NO: 37 - DNA, 40 bp, synthetic construct
  misc_feature 1..40: note = synthetic primer
  source 1..40: mol_type = other DNA
cggcgctggcgtcgtggtacgtttgatctccagcttggtg

SEQ ID NO: 38 - DNA, 765 bp, synthetic construct
  misc_feature 1..765: note = synthetic polynucleotide
  source 1..765: mol_type = other DNA
ctccacgccgccaggccggaggtgcagctggtgcagagcggcgccgaggtgaagaagcccggcgccagcgtgaaggtgagctgcaaggccagcggctacaccttcagcgactacgagatgcactgggtgcggcaggcccccggccagggcctggagtggatgggcgccatccaccccggcagcggcgacaccgcctacaaccagcggttcaagggccgggtgaccatcaccgccgacaagagcaccagcaccgcctacatggagctgagcagcctgcggagcgaggacaccgccgtgtactactgcgcccggttctacagctacgcctactggggccagggcaccctggtgaccgtgagcgccggtggaggcggttcaggcggaggtggttctggcggtggcggatcggacatcgtgatgacccagacccccctgagcctgcccgtgacccccggcgagcccgccagcatcagctgccggagcagccagagcctggtgcacagcaacggcaacacctacctgcagtggtacctgcagaagcccggccagagcccccagctgctgatctacaaggtgagcaaccggttcagcggcgtgcccgaccggttcagcggcagcggcagcggcaccgacttcaccctgaagatcagccgggtggaggccgaggacgtgggcgtgtactactgcagccagagcatctacgtgccctacaccttcggccagggcaccaagctggagatcaaacgtaccacgacgccagcgccg

SEQ ID NO: 39 - DNA, 18 bp, synthetic construct
  misc_feature 1..18: note = synthetic primer
  source 1..18: mol_type = other DNA
accacgacgccagcgccg

SEQ ID NO: 40 - DNA, 44 bp, synthetic construct
  misc_feature 1..44: note = synthetic primer
  source 1..44: mol_type = other DNA
aatccagaggttgattgtcgacctagcgagggggcagggcctgc

SEQ ID NO: 41 - DNA, 703 bp, synthetic construct
  misc_feature 1..703: note = synthetic polynucleotide
  source 1..703: mol_type = other DNA
accacgacgccagcgccgcgaccaccaacaccggcgcccaccatcgcgtcgcagcccctgtccctgcgcccagaggcgtgccggccagcggcggggggcgcagtgcacacgagggggctggacttcgcctgtgatttttgggtgctggtggtggttggtggagtcctggcttgctatagcttgctagtaacagtggcctttattattttctgggtgaggagtaagaggagcaggctcctgcacagtgactacatgaacatgactccccgccgccccgggccaacccgcaagcattaccagccctatgccccaccacgcgacttcgcagcctatcgctccagagtgaagttcagcaggagcgcagacgcccccgcgtaccagcagggccagaaccagctctataacgagctcaatctaggacgaagagaggagtacgatgttttggacaagagacgtggccgggaccctgagatggggggaaagccgcagagaaggaagaaccctcaggaaggcctgtacaatgaactgcagaaagataagatggcggaggcctacagtgagattgggatgaaaggcgagcgccggaggggcaaggggcacgatggcctttaccagggtctcagtacagccaccaaggacacctacgacgcccttcacatgcaggccctgccccctcgctaggtcgacaatcaacctctggatt